European Patent Specification EP 3 690 064 B1, published September 6, 2023. Title: A method for distinguishing onions. Applicant: House Foods Group Inc. The sequence listing filed with the application follows.

SEQUENCE LISTING (22 sequences)

SEQ ID NO: 1 - DNA, 1663 bp, Allium cepa
ccgagattacaagtggagcattaaatatccatagcagagctaattagctatggagtcttaccacaaagttggcagtaataaaatgccaagccttcttattttgatatgcataatcatgtcttcatttgttaacaataatatagctcaagcgaaggtgacatggagtttgaaggcagcagaagaggcagaagcagtggctaatataaactgttcagggcatgggagagcttttttggacggaattctttcagatggatctcctaaatgcgagtgcaatacttgctacactggtgcagactgctctgaaaagattacaggttgctctgctgatgttgccagtggtgatggactgtttctagaagaatactggcagcagcacaaggaaaacagtgcagtgctggtttcaggatggcacagaatgagctactttttcaacccagttagcaatttcatatctttcgagcttgaaaaaacaattaaagaactacatgagatagtcggaaatgctgctgcaaaggacaggtacattgtgtttggagtaggggtgactcaactcatccatggattggtcatctctctttcaccaaatatgactgccactccttgtgcaccacaatctaaagttgttgctcatgccccttattatccggtgtttagagaacaaacaaagtactttgacaagaaagggtacgagtggaaaggaaatgcagcggattacgtgaacacttcaactccagagcaattcattgagatggttacttcacctaataacccagaaggtctgcttcgccatgaagtaataaagggatgcaaatccatctacgatatggtttactactggcctcattacaccccaatcaagtacaaagccgatgaagatatcatgttgtttacaatgtctaaatacactggacactctggtagtcgatttgggtgggcactgataaaggatgaaactgtgtataataaattgttgaattacatgacaaagaacacggagggcacttcccgagaaacacagctacgatcgctcaaaattctaaaagaagttatagcaatggttaaaacacagaaaggcaccatgcgcgacctcaacacatttggttttcagaaactaagagagaggtgggtaaatatcacttcattgctcgataaatccgacagattctcctatcaaaagcttccacaaagtgaatattgcaattacttcaggagaatgagacctccatccccatcttatgcatgggtgaagtgtgaatgggaagaagacaaagattgctaccagacatttcaaaatgggcgtatcaatacgcaaagtggagagggtttcgaagcaggtagtcgttatgtgcgtttgagtttgatcaagacaaaagatgattttgatcaactaatgtactatttgaagaatatggttgaagcaaagaggaagactcctctcatcaaacaactttccaatgatcagatctcccgccgtcctttcatttaagtactcatgttatgtattgctctgctgttttgttagtgtatgactatgttcatacatcctaatgctatggtagtaaggagtatctttctatgcaataaataaagttcatgtttgtgatcatgtatgggctactatgattttataataaaatcaattttcatataaaaaaaaaaa

SEQ ID NO: 2 - DNA, 1975 bp, Allium cepa
ccacaaagttggcagtagtaaaatgccaagcctacttattttgatatgcataatcatgtcttcatttgtcaacaataatatagctcaagggaaggtgacatggagtttgaaggcagcagaagaggcggaggcagtggccaatataaactgttcagggcatggaagagcttttttggatggaattctttcagatggctctcctaaatgcgagtgcaatacttgctacactggtgcagattgctctcaaaagattacaggttgctctgcggatgttgccaggttaatatttctctgttcttcacaatacatggtagtttaactttatatcaaacacactggacaatatttaatgacatgcttaaggaattgaatgatatattgtatacacagtgstgatggactgwttcttgaggaatattggcagcascacmaggaaaacagtgcagtgctcgtttcaggatggcacagaatgagctactttttcaacccagytagcaatttcatatcgttcgagcttgaaaaaacaattaaggaactacatgagatagtcggaaatgctgctgcaaaggacaggtacattgtgtttggagtcggggtgactcaactcatccatggattggtcatctytctttcaccaaatatgactgccactccttgtgcaccacaatctaaagttgttgctcatgcccctttttatccggtaactctacgcatgtttctaagttgaactacctagagataactgtttatttcttatgtactcgtgtgactgacttaatttgaacaaattaaatgatacaggtgttcagagaacaaacaaaatattttgacaagaaagggtacgagtggaaaggaaatgcagcgaattacgtgaacacttcaactcctgagcagttcattgagatggttacttcacctaataacccagaaggtctgcttcgcaaggaagtaatcaagggatgcaaatccatttacgatatggtttactactggcctcattacaccccaatcaagtacaaagccgacgaagatatcatgttgtttacaatgtctaaatacactggacactctggtagtcgatttgggtatgtccacatattattacctcacatctttctctacctataattaacatatttaagttggttagttagtaactcatactttaatatcttattaaattaggtgggcgttgataaaggatgaaaccgtgtataataagttgtwaaattacatgacaaaaaacacggaaggcactcctcgggaaacacagctacgatcgctcaaaattmtaaaagaagtcatagcaatggttaaaacacagaaaggcaccatgcgtgacctcaacacatttggttttaagaaactaagagagaggtgggtaaatatcactgcattgctggataaatcagacagattctcctatcaaaagcttccacaaagtgaatattgcaattacttccgaagaatgagacctccatccccatgtatgtataccagtatattatcatttattgaaagatataatattatagattataaacataacaatgyagcattaatcaatgatatatatatacacgatgacagcttatgcatgggtgaagtgtgaatgggaagaagacaaagattgctaccagacatttcaaaatggacgyatcaacacacaaagtggagagggtttcgaagcgggcagtcgttacgtgcgtytgagtttgatcaagacaaaggatgattttgatcaactcatgtactatttgaagactatggttgaagcaaagaggaagactcctctcatcaaacaactttccaatgatcagacatcccgccgtcctttcatttaagtactcatgttatgtatcgctcgctgttttgttagtgtatgactatgttcatacatcctaatgctatggtcgtaaggagttcctatctttgtaataaataaagttcatgtttgtgatcatgtatggrctac

SEQ ID NO: 3 - DNA, 27 bp, Artificial
  Primer
atggagtcttaccacaaagttggcagt

SEQ ID NO: 4 - DNA, 29 bp, Artificial
  Primer
gtagcccatacatgatcacaaacatgaac

SEQ ID NO: 5 - DNA, 25 bp, Artificial
  Primer
tggcagtaataaaatgccaagcctt

SEQ ID NO: 6 - DNA, 25 bp, Artificial
  Primer
atgcataatcatgtcttcatttgtt

SEQ ID NO: 7 - DNA, 30 bp, Artificial
  Primer
cagacatttcaaaatgggcgtatcaatacg

SEQ ID NO: 8 - DNA, 29 bp, Artificial
  Primer
gagagggtttcgaagcaggtagtcgttat

SEQ ID NO: 9 - DNA, 25 bp, Artificial
  Primer
acagtttatattagccactgcttct

SEQ ID NO: 10 - DNA, 23 bp, Artificial
  Primer
tgtgctgctgccagtattcttct

SEQ ID NO: 11 - DNA, 25 bp, Artificial
  Primer
atttgcatccctttattacttcatg

SEQ ID NO: 12 - DNA, 27 bp, Artificial
  Primer
gtacttaaatgaaaggacggcgggaga

SEQ ID NO: 13 - DNA, 25 bp, Artificial
  Primer
tggcagtagtaaaatgccaagccta

SEQ ID NO: 14 - DNA, 25 bp, Artificial
  Primer
atgcataatcatgtcttcatttgtc

SEQ ID NO: 15 - DNA, 30 bp, Artificial
  Primer
cagacatttcaaaatggacgyatcaacaca

SEQ ID NO: 16 - DNA, 29 bp, Artificial
  Primer
gagagggtttcgaagcgggcagtcgttac

SEQ ID NO: 17 - DNA, 25 bp, Artificial
  Primer
acagtttatattggccactgcctcc

SEQ ID NO: 18 - DNA, 23 bp, Artificial
  Primer
ggtggtgctgccaatattcctca

SEQ ID NO: 19 - DNA, 29 bp, Artificial
  Primer
atggatttgcatcccttgattacttcctt

SEQ ID NO: 20 - DNA, 27 bp, Artificial
  Primer
gtacttaaatgaaaggacggcgggatg

SEQ ID NO: 21 - DNA, 28 bp, Artificial
  Primer
atatggtttactactggcctcattacac

SEQ ID NO: 22 - DNA, 26 bp, Artificial
  Primer
ccattcacacttcacccatgcataag